European Patent Application EP 4 628 510 A1, published October 8, 2025. Title: 痘病毒多抗原嵌合疫苗及其用途. Applicant: 中国科学院微生物研究所. The sequence listing filed with the application follows.

SEQUENCE LISTING (27 sequences)

SEQ ID NO: 1 - protein, 92 aa, synthetic construct
STTQYDHKESCNGLYYQGSCYILHSDYKSFEDAKANCAAESSTLPNKSDVLTTWLIDYVEDTWGSDGNPITKTTSDYQDSDVSQEVRKYFCT

SEQ ID NO: 2 - protein, 118 aa, synthetic construct
SANKAAITDSAVAVAAASSTHRKVVSSTTQYDHKESCNGLYYQGSCYILHSDYKSFEDAKANCAAESSTLPNKSDVLTTWLIDYVEDTWGSDGNPITKTTSDYQDSDVSQEVRKYFCT

SEQ ID NO: 3 - protein, 179 aa, synthetic construct
AAASIQTTVNTLSERISSKLEQEANASAQTKCDIEIGNFYIRQNHGCNITVKNMCSADADAQLDAVLSAATETYSGLTPEQKAYVPAMFTAALNIQTSVNTVVRDFENYVKQTCNSSAVVDNKLKIQNVIIDECYGAPGSPTNLEFINTGSSKGNCAIKALMQLTTKATTQIAPRQVAG

SEQ ID NO: 4 - protein, 260 aa, synthetic construct
TCTVPTMNNAKLTSTETSFNDKQKVTFTCDSGYHSLDPNAVCETDKWKYENPCKKMCTVSDYVSELYDKPLYEVNSTMTLSCNGETKYFRCEEKNGNTSWNDTVTCPNAECQPLQLEHGSCQPVKEKYSFGEYMTINCDVGYEVIGVSYISCTANSWNVIPSCQQKCDIPSLSNGLISGSTFSIGGVIHLSCKSGFTLTGSPSSTCIDGKWNPILPTCVRSNEEFDPVDDGPDDETDLSKLSKDVVQYEQEIESLEATYH

SEQ ID NO: 5 - protein, 260 aa, synthetic construct
TCTVPTMNNAKLTSTETSFNDKQKVTFTCDSGYHSLDPNAVCETDKWKYENPCKKMCTVSDYVSELYDKPLYEVNSTMTLSCNGETKYFRCEEKNGNTSWNDTVTCPNAECQPLQLEHGSSQPVKEKYSFGEYMTINCDVGYEVIGVSYISCTANSWNVIPSCQQKCDIPSLSNGLISGSTFSIGGVIHLSCKSGFTLTGSPSSTCIDGKWNPILPTCVRSNEEFDPVDDGPDDETDLSKLSKDVVQYEQEIESLEATYH

SEQ ID NO: 6 - protein, 649 aa, synthetic construct
STTQYDHKESCNGLYYQGSCYILHSDYKSFEDAKANCAAESSTLPNKSDVLTTWLIDYVEDTWGSDGNPITKTTSDYQDSDVSQEVRKYFCTAAASIQTTVNTLSERISSKLEQEANASAQTKCDIEIGNFYIRQNHGCNITVKNMCSADADAQLDAVLSAATETYSGLTPEQKAYVPAMFTAALNIQTSVNTVVRDFENYVKQTCNSSAVVDNKLKIQNVIIDECYGAPGSPTNLEFINTGSSKGNCAIKALMQLTTKATTQIAPRQVAGSANKAAITDSAVAVAAASSTHRKVVSSTTQYDHKESCNGLYYQGSCYILHSDYKSFEDAKANCAAESSTLPNKSDVLTTWLIDYVEDTWGSDGNPITKTTSDYQDSDVSQEVRKYFCTTCTVPTMNNAKLTSTETSFNDKQKVTFTCDSGYHSLDPNAVCETDKWKYENPCKKMCTVSDYVSELYDKPLYEVNSTMTLSCNGETKYFRCEEKNGNTSWNDTVTCPNAECQPLQLEHGSCQPVKEKYSFGEYMTINCDVGYEVIGVSYISCTANSWNVIPSCQQKCDIPSLSNGLISGSTFSIGGVIHLSCKSGFTLTGSPSSTCIDGKWNPILPTCVRSNEEFDPVDDGPDDETDLSKLSKDVVQYEQEIESLEATYH

SEQ ID NO: 7 - protein, 649 aa, synthetic construct
STTQYDHKESCNGLYYQGSCYILHSDYKSFEDAKANCAAESSTLPNKSDVLTTWLIDYVEDTWGSDGNPITKTTSDYQDSDVSQEVRKYFCTAAASIQTTVNTLSERISSKLEQEANASAQTKCDIEIGNFYIRQNHGCNITVKNMCSADADAQLDAVLSAATETYSGLTPEQKAYVPAMFTAALNIQTSVNTVVRDFENYVKQTCNSSAVVDNKLKIQNVIIDECYGAPGSPTNLEFINTGSSKGNCAIKALMQLTTKATTQIAPRQVAGSANKAAITDSAVAVAAASSTHRKVVSSTTQYDHKESCNGLYYQGSCYILHSDYKSFEDAKANCAAESSTLPNKSDVLTTWLIDYVEDTWGSDGNPITKTTSDYQDSDVSQEVRKYFCTTCTVPTMNNAKLTSTETSFNDKQKVTFTCDSGYHSLDPNAVCETDKWKYENPCKKMCTVSDYVSELYDKPLYEVNSTMTLSCNGETKYFRCEEKNGNTSWNDTVTCPNAECQPLQLEHGSSQPVKEKYSFGEYMTINCDVGYEVIGVSYISCTANSWNVIPSCQQKCDIPSLSNGLISGSTFSIGGVIHLSCKSGFTLTGSPSSTCIDGKWNPILPTCVRSNEEFDPVDDGPDDETDLSKLSKDVVQYEQEIESLEATYH

SEQ ID NO: 8 - protein, 531 aa, synthetic construct
STTQYDHKESCNGLYYQGSCYILHSDYKSFEDAKANCAAESSTLPNKSDVLTTWLIDYVEDTWGSDGNPITKTTSDYQDSDVSQEVRKYFCTAAASIQTTVNTLSERISSKLEQEANASAQTKCDIEIGNFYIRQNHGCNITVKNMCSADADAQLDAVLSAATETYSGLTPEQKAYVPAMFTAALNIQTSVNTVVRDFENYVKQTCNSSAVVDNKLKIQNVIIDECYGAPGSPTNLEFINTGSSKGNCAIKALMQLTTKATTQIAPRQVAGTCTVPTMNNAKLTSTETSFNDKQKVTFTCDSGYHSLDPNAVCETDKWKYENPCKKMCTVSDYVSELYDKPLYEVNSTMTLSCNGETKYFRCEEKNGNTSWNDTVTCPNAECQPLQLEHGSCQPVKEKYSFGEYMTINCDVGYEVIGVSYISCTANSWNVIPSCQQKCDIPSLSNGLISGSTFSIGGVIHLSCKSGFTLTGSPSSTCIDGKWNPILPTCVRSNEEFDPVDDGPDDETDLSKLSKDVVQYEQEIESLEATYH

SEQ ID NO: 9 - protein, 531 aa, synthetic construct
STTQYDHKESCNGLYYQGSCYILHSDYKSFEDAKANCAAESSTLPNKSDVLTTWLIDYVEDTWGSDGNPITKTTSDYQDSDVSQEVRKYFCTAAASIQTTVNTLSERISSKLEQEANASAQTKCDIEIGNFYIRQNHGCNITVKNMCSADADAQLDAVLSAATETYSGLTPEQKAYVPAMFTAALNIQTSVNTVVRDFENYVKQTCNSSAVVDNKLKIQNVIIDECYGAPGSPTNLEFINTGSSKGNCAIKALMQLTTKATTQIAPRQVAGTCTVPTMNNAKLTSTETSFNDKQKVTFTCDSGYHSLDPNAVCETDKWKYENPCKKMCTVSDYVSELYDKPLYEVNSTMTLSCNGETKYFRCEEKNGNTSWNDTVTCPNAECQPLQLEHGSSQPVKEKYSFGEYMTINCDVGYEVIGVSYISCTANSWNVIPSCQQKCDIPSLSNGLISGSTFSIGGVIHLSCKSGFTLTGSPSSTCIDGKWNPILPTCVRSNEEFDPVDDGPDDETDLSKLSKDVVQYEQEIESLEATYH

SEQ ID NO: 10 - DNA, 1947 bp, synthetic construct
  source 1..1947: mol_type = other DNA
agcaccacccagtacgaccacaaagagagctgcaacggcctgtactaccaaggctcttgttacatcctgcacagcgactataagagcttcgaggatgctaaggccaattgcgccgccgagagcagcacactgcctaacaagtccgacgtgctgaccacctggctgatcgactacgtggaagatacatggggaagcgacggcaaccccatcacaaaaaccacaagcgattatcaggacagcgacgtgtctcaggaggttagaaagtacttttgcaccgccgccgcctctatccagaccacagtgaacaccctgagcgagcggatcagctccaagctggagcaggaggcaaacgcaagcgcccagacaaagtgcgacatcgagatcggcaatttctacatcagacagaaccacggctgcaatatcaccgtgaagaatatgtgctccgccgacgcagatgcacagctggatgccgtgctgtccgccgcaaccgagacatactctggcctgacccctgagcagaaggcctatgtgccagccatgttcacagccgccctgaacatccagaccagcgtgaatacagtggtgcgggactttgagaactacgtgaagcagacctgcaattctagcgccgtggtggacaacaagctgaagatccagaatgtgatcatcgatgagtgttatggagcaccaggctcccctaccaacctggagttcatcaatacaggctcctctaagggcaactgcgccatcaaggccctgatgcagctgaccacaaaggccaccacacagatcgcacctaggcaggtggcaggctccgccaataaggcagccatcaccgactctgccgtggcagtggcagcagccagctccacacaccgcaaggtggtgtctagcaccacacagtacgatcacaaggaatcctgtaatggcctgtactatcagggctcctgttacatcctgcactctgactataagagctttgaggatgccaaggccaactgtgccgccgagtcctctaccctgccaaataagagcgacgtgctgaccacatggctgatcgactatgtggaggatacctggggctctgatggcaaccccatcacaaagaccacatctgattaccaggacagcgacgtgagccaggaggtgcggaagtatttctgcaccacgtgcacggtgcccacgatgaacaacgcgaagttgacgtccacggaaacctctttcaatgataaacaaaaagtcacgttcacatgtgactccggataccactctttggacccgaacgcagtttgtgaaacagataagtggaagtacgagaatccgtgcaagaaaatgtgcacggtgtcggattatgtatcagagttgtacgacaagccgttgtacgaggttaatagtaccatgaccttgtcgtgcaacggcgaaaccaagtatttccgttgtgaagagaaaaacgggaacacgtcgtggaacgacacggtaacctgccccaacgcggagtgtcaacctctgcagttggagcacggctcttgtcagccggtgaaggaaaaatattccttcggcgagtacatgactataaactgtgatgtggggtacgaggttataggcgtatcctacattagctgcaccgctaatagttggaacgtcatcccctcgtgccagcagaaatgcgacattccgtctctgtcaaatggcctgatctccgggtcgaccttctcgataggtggggttattcatttgtcctgtaagagtgggttcactcttacaggctccccatcttcgacctgcatagatgggaagtggaaccccatccttcccacttgtgtcaggtcgaacgaggaattcgatccggtagatgacggccctgacgacgagacggatctgtcgaagctgtccaaagacgtggttcagtatgagcaggagatagaatctcttgaggctacttaccac

SEQ ID NO: 11 - DNA, 1947 bp, synthetic construct
  source 1..1947: mol_type = other DNA
agcaccacccagtacgaccacaaagagagctgcaacggcctgtactaccaaggctcttgttacatcctgcacagcgactataagagcttcgaggatgctaaggccaattgcgccgccgagagcagcacactgcctaacaagtccgacgtgctgaccacctggctgatcgactacgtggaagatacatggggaagcgacggcaaccccatcacaaaaaccacaagcgattatcaggacagcgacgtgtctcaggaggttagaaagtacttttgcaccgccgccgcctctatccagaccacagtgaacaccctgagcgagcggatcagctccaagctggagcaggaggcaaacgcaagcgcccagacaaagtgcgacatcgagatcggcaatttctacatcagacagaaccacggctgcaatatcaccgtgaagaatatgtgctccgccgacgcagatgcacagctggatgccgtgctgtccgccgcaaccgagacatactctggcctgacccctgagcagaaggcctatgtgccagccatgttcacagccgccctgaacatccagaccagcgtgaatacagtggtgcgggactttgagaactacgtgaagcagacctgcaattctagcgccgtggtggacaacaagctgaagatccagaatgtgatcatcgatgagtgttatggagcaccaggctcccctaccaacctggagttcatcaatacaggctcctctaagggcaactgcgccatcaaggccctgatgcagctgaccacaaaggccaccacacagatcgcacctaggcaggtggcaggctccgccaataaggcagccatcaccgactctgccgtggcagtggcagcagccagctccacacaccgcaaggtggtgtctagcaccacacagtacgatcacaaggaatcctgtaatggcctgtactatcagggctcctgttacatcctgcactctgactataagagctttgaggatgccaaggccaactgtgccgccgagtcctctaccctgccaaataagagcgacgtgctgaccacatggctgatcgactatgtggaggatacctggggctctgatggcaaccccatcacaaagaccacatctgattaccaggacagcgacgtgagccaggaggtgcggaagtatttctgcaccacgtgcacggtgcccacgatgaacaacgcgaagttgacgtccacggaaacctctttcaatgataaacaaaaagtcacgttcacatgtgactccggataccactctttggacccgaacgcagtttgtgaaacagataagtggaagtacgagaatccgtgcaagaaaatgtgcacggtgtcggattatgtatcagagttgtacgacaagccgttgtacgaggttaatagtaccatgaccttgtcgtgcaacggcgaaaccaagtatttccgttgtgaagagaaaaacgggaacacgtcgtggaacgacacggtaacctgccccaacgcggagtgtcaacctctgcagttggagcacggctcttctcagccggtgaaggaaaaatattccttcggcgagtacatgactataaactgtgatgtggggtacgaggttataggcgtatcctacattagctgcaccgctaatagttggaacgtcatcccctcgtgccagcagaaatgcgacattccgtctctgtcaaatggcctgatctccgggtcgaccttctcgataggtggggttattcatttgtcctgtaagagtgggttcactcttacaggctccccatcttcgacctgcatagatgggaagtggaaccccatccttcccacttgtgtcaggtcgaacgaggaattcgatccggtagatgacggccctgacgacgagacggatctgtcgaagctgtccaaagacgtggttcagtatgagcaggagatagaatctcttgaggctacttaccac

SEQ ID NO: 12 - DNA, 1593 bp, synthetic construct
  source 1..1593: mol_type = other DNA
agcaccacccagtacgaccacaaagagagctgcaacggcctgtactaccaaggctcttgttacatcctgcacagcgactataagagcttcgaggatgctaaggccaattgcgccgccgagagcagcacactgcctaacaagtccgacgtgctgaccacctggctgatcgactacgtggaagatacatggggaagcgacggcaaccccatcacaaaaaccacaagcgattatcaggacagcgacgtgtctcaggaggttagaaagtacttttgcaccgccgccgcctctatccagaccacagtgaacaccctgagcgagcggatcagctccaagctggagcaggaggcaaacgcaagcgcccagacaaagtgcgacatcgagatcggcaatttctacatcagacagaaccacggctgcaatatcaccgtgaagaatatgtgctccgccgacgcagatgcacagctggatgccgtgctgtccgccgcaaccgagacatactctggcctgacccctgagcagaaggcctatgtgccagccatgttcacagccgccctgaacatccagaccagcgtgaatacagtggtgcgggactttgagaactacgtgaagcagacctgcaattctagcgccgtggtggacaacaagctgaagatccagaatgtgatcatcgatgagtgttatggagcaccaggctcccctaccaacctggagttcatcaatacaggctcctctaagggcaactgcgccatcaaggccctgatgcagctgaccacaaaggccaccacacagatcgcacctaggcaggtggcaggcacgtgcacggtgcccacgatgaacaacgcgaagttgacgtccacggaaacctctttcaatgataaacaaaaagtcacgttcacatgtgactccggataccactctttggacccgaacgcagtttgtgaaacagataagtggaagtacgagaatccgtgcaagaaaatgtgcacggtgtcggattatgtatcagagttgtacgacaagccgttgtacgaggttaatagtaccatgaccttgtcgtgcaacggcgaaaccaagtatttccgttgtgaagagaaaaacgggaacacgtcgtggaacgacacggtaacctgccccaacgcggagtgtcaacctctgcagttggagcacggctcttgtcagccggtgaaggaaaaatattccttcggcgagtacatgactataaactgtgatgtggggtacgaggttataggcgtatcctacattagctgcaccgctaatagttggaacgtcatcccctcgtgccagcagaaatgcgacattccgtctctgtcaaatggcctgatctccgggtcgaccttctcgataggtggggttattcatttgtcctgtaagagtgggttcactcttacaggctccccatcttcgacctgcatagatgggaagtggaaccccatccttcccacttgtgtcaggtcgaacgaggaattcgatccggtagatgacggccctgacgacgagacggatctgtcgaagctgtccaaagacgtggttcagtatgagcaggagatagaatctcttgaggctacttaccac

SEQ ID NO: 13 - DNA, 1593 bp, synthetic construct
  source 1..1593: mol_type = other DNA
agcaccacccagtacgaccacaaagagagctgcaacggcctgtactaccaaggctcttgttacatcctgcacagcgactataagagcttcgaggatgctaaggccaattgcgccgccgagagcagcacactgcctaacaagtccgacgtgctgaccacctggctgatcgactacgtggaagatacatggggaagcgacggcaaccccatcacaaaaaccacaagcgattatcaggacagcgacgtgtctcaggaggttagaaagtacttttgcaccgccgccgcctctatccagaccacagtgaacaccctgagcgagcggatcagctccaagctggagcaggaggcaaacgcaagcgcccagacaaagtgcgacatcgagatcggcaatttctacatcagacagaaccacggctgcaatatcaccgtgaagaatatgtgctccgccgacgcagatgcacagctggatgccgtgctgtccgccgcaaccgagacatactctggcctgacccctgagcagaaggcctatgtgccagccatgttcacagccgccctgaacatccagaccagcgtgaatacagtggtgcgggactttgagaactacgtgaagcagacctgcaattctagcgccgtggtggacaacaagctgaagatccagaatgtgatcatcgatgagtgttatggagcaccaggctcccctaccaacctggagttcatcaatacaggctcctctaagggcaactgcgccatcaaggccctgatgcagctgaccacaaaggccaccacacagatcgcacctaggcaggtggcaggcacgtgcacggtgcccacgatgaacaacgcgaagttgacgtccacggaaacctctttcaatgataaacaaaaagtcacgttcacatgtgactccggataccactctttggacccgaacgcagtttgtgaaacagataagtggaagtacgagaatccgtgcaagaaaatgtgcacggtgtcggattatgtatcagagttgtacgacaagccgttgtacgaggttaatagtaccatgaccttgtcgtgcaacggcgaaaccaagtatttccgttgtgaagagaaaaacgggaacacgtcgtggaacgacacggtaacctgccccaacgcggagtgtcaacctctgcagttggagcacggctcttctcagccggtgaaggaaaaatattccttcggcgagtacatgactataaactgtgatgtggggtacgaggttataggcgtatcctacattagctgcaccgctaatagttggaacgtcatcccctcgtgccagcagaaatgcgacattccgtctctgtcaaatggcctgatctccgggtcgaccttctcgataggtggggttattcatttgtcctgtaagagtgggttcactcttacaggctccccatcttcgacctgcatagatgggaagtggaaccccatccttcccacttgtgtcaggtcgaacgaggaattcgatccggtagatgacggccctgacgacgagacggatctgtcgaagctgtccaaagacgtggttcagtatgagcaggagatagaatctcttgaggctacttaccac

SEQ ID NO: 14 - RNA, 1947 nt, synthetic construct
  source 1..1947: mol_type = other RNA
agcaccacccagtacgaccacaaagagagctgcaacggcctgtactaccaaggctcttgttacatcctgcacagcgactataagagcttcgaggatgctaaggccaattgcgccgccgagagcagcacactgcctaacaagtccgacgtgctgaccacctggctgatcgactacgtggaagatacatggggaagcgacggcaaccccatcacaaaaaccacaagcgattatcaggacagcgacgtgtctcaggaggttagaaagtacttttgcaccgccgccgcctctatccagaccacagtgaacaccctgagcgagcggatcagctccaagctggagcaggaggcaaacgcaagcgcccagacaaagtgcgacatcgagatcggcaatttctacatcagacagaaccacggctgcaatatcaccgtgaagaatatgtgctccgccgacgcagatgcacagctggatgccgtgctgtccgccgcaaccgagacatactctggcctgacccctgagcagaaggcctatgtgccagccatgttcacagccgccctgaacatccagaccagcgtgaatacagtggtgcgggactttgagaactacgtgaagcagacctgcaattctagcgccgtggtggacaacaagctgaagatccagaatgtgatcatcgatgagtgttatggagcaccaggctcccctaccaacctggagttcatcaatacaggctcctctaagggcaactgcgccatcaaggccctgatgcagctgaccacaaaggccaccacacagatcgcacctaggcaggtggcaggctccgccaataaggcagccatcaccgactctgccgtggcagtggcagcagccagctccacacaccgcaaggtggtgtctagcaccacacagtacgatcacaaggaatcctgtaatggcctgtactatcagggctcctgttacatcctgcactctgactataagagctttgaggatgccaaggccaactgtgccgccgagtcctctaccctgccaaataagagcgacgtgctgaccacatggctgatcgactatgtggaggatacctggggctctgatggcaaccccatcacaaagaccacatctgattaccaggacagcgacgtgagccaggaggtgcggaagtatttctgcaccacgtgcacggtgcccacgatgaacaacgcgaagttgacgtccacggaaacctctttcaatgataaacaaaaagtcacgttcacatgtgactccggataccactctttggacccgaacgcagtttgtgaaacagataagtggaagtacgagaatccgtgcaagaaaatgtgcacggtgtcggattatgtatcagagttgtacgacaagccgttgtacgaggttaatagtaccatgaccttgtcgtgcaacggcgaaaccaagtatttccgttgtgaagagaaaaacgggaacacgtcgtggaacgacacggtaacctgccccaacgcggagtgtcaacctctgcagttggagcacggctcttgtcagccggtgaaggaaaaatattccttcggcgagtacatgactataaactgtgatgtggggtacgaggttataggcgtatcctacattagctgcaccgctaatagttggaacgtcatcccctcgtgccagcagaaatgcgacattccgtctctgtcaaatggcctgatctccgggtcgaccttctcgataggtggggttattcatttgtcctgtaagagtgggttcactcttacaggctccccatcttcgacctgcatagatgggaagtggaaccccatccttcccacttgtgtcaggtcgaacgaggaattcgatccggtagatgacggccctgacgacgagacggatctgtcgaagctgtccaaagacgtggttcagtatgagcaggagatagaatctcttgaggctacttaccac

SEQ ID NO: 15 - RNA, 1947 nt, synthetic construct
  source 1..1947: mol_type = other RNA
agcaccacccagtacgaccacaaagagagctgcaacggcctgtactaccaaggctcttgttacatcctgcacagcgactataagagcttcgaggatgctaaggccaattgcgccgccgagagcagcacactgcctaacaagtccgacgtgctgaccacctggctgatcgactacgtggaagatacatggggaagcgacggcaaccccatcacaaaaaccacaagcgattatcaggacagcgacgtgtctcaggaggttagaaagtacttttgcaccgccgccgcctctatccagaccacagtgaacaccctgagcgagcggatcagctccaagctggagcaggaggcaaacgcaagcgcccagacaaagtgcgacatcgagatcggcaatttctacatcagacagaaccacggctgcaatatcaccgtgaagaatatgtgctccgccgacgcagatgcacagctggatgccgtgctgtccgccgcaaccgagacatactctggcctgacccctgagcagaaggcctatgtgccagccatgttcacagccgccctgaacatccagaccagcgtgaatacagtggtgcgggactttgagaactacgtgaagcagacctgcaattctagcgccgtggtggacaacaagctgaagatccagaatgtgatcatcgatgagtgttatggagcaccaggctcccctaccaacctggagttcatcaatacaggctcctctaagggcaactgcgccatcaaggccctgatgcagctgaccacaaaggccaccacacagatcgcacctaggcaggtggcaggctccgccaataaggcagccatcaccgactctgccgtggcagtggcagcagccagctccacacaccgcaaggtggtgtctagcaccacacagtacgatcacaaggaatcctgtaatggcctgtactatcagggctcctgttacatcctgcactctgactataagagctttgaggatgccaaggccaactgtgccgccgagtcctctaccctgccaaataagagcgacgtgctgaccacatggctgatcgactatgtggaggatacctggggctctgatggcaaccccatcacaaagaccacatctgattaccaggacagcgacgtgagccaggaggtgcggaagtatttctgcaccacgtgcacggtgcccacgatgaacaacgcgaagttgacgtccacggaaacctctttcaatgataaacaaaaagtcacgttcacatgtgactccggataccactctttggacccgaacgcagtttgtgaaacagataagtggaagtacgagaatccgtgcaagaaaatgtgcacggtgtcggattatgtatcagagttgtacgacaagccgttgtacgaggttaatagtaccatgaccttgtcgtgcaacggcgaaaccaagtatttccgttgtgaagagaaaaacgggaacacgtcgtggaacgacacggtaacctgccccaacgcggagtgtcaacctctgcagttggagcacggctcttctcagccggtgaaggaaaaatattccttcggcgagtacatgactataaactgtgatgtggggtacgaggttataggcgtatcctacattagctgcaccgctaatagttggaacgtcatcccctcgtgccagcagaaatgcgacattccgtctctgtcaaatggcctgatctccgggtcgaccttctcgataggtggggttattcatttgtcctgtaagagtgggttcactcttacaggctccccatcttcgacctgcatagatgggaagtggaaccccatccttcccacttgtgtcaggtcgaacgaggaattcgatccggtagatgacggccctgacgacgagacggatctgtcgaagctgtccaaagacgtggttcagtatgagcaggagatagaatctcttgaggctacttaccac

SEQ ID NO: 16 - RNA, 1593 nt, synthetic construct
  source 1..1593: mol_type = other RNA
agcaccacccagtacgaccacaaagagagctgcaacggcctgtactaccaaggctcttgttacatcctgcacagcgactataagagcttcgaggatgctaaggccaattgcgccgccgagagcagcacactgcctaacaagtccgacgtgctgaccacctggctgatcgactacgtggaagatacatggggaagcgacggcaaccccatcacaaaaaccacaagcgattatcaggacagcgacgtgtctcaggaggttagaaagtacttttgcaccgccgccgcctctatccagaccacagtgaacaccctgagcgagcggatcagctccaagctggagcaggaggcaaacgcaagcgcccagacaaagtgcgacatcgagatcggcaatttctacatcagacagaaccacggctgcaatatcaccgtgaagaatatgtgctccgccgacgcagatgcacagctggatgccgtgctgtccgccgcaaccgagacatactctggcctgacccctgagcagaaggcctatgtgccagccatgttcacagccgccctgaacatccagaccagcgtgaatacagtggtgcgggactttgagaactacgtgaagcagacctgcaattctagcgccgtggtggacaacaagctgaagatccagaatgtgatcatcgatgagtgttatggagcaccaggctcccctaccaacctggagttcatcaatacaggctcctctaagggcaactgcgccatcaaggccctgatgcagctgaccacaaaggccaccacacagatcgcacctaggcaggtggcaggcacgtgcacggtgcccacgatgaacaacgcgaagttgacgtccacggaaacctctttcaatgataaacaaaaagtcacgttcacatgtgactccggataccactctttggacccgaacgcagtttgtgaaacagataagtggaagtacgagaatccgtgcaagaaaatgtgcacggtgtcggattatgtatcagagttgtacgacaagccgttgtacgaggttaatagtaccatgaccttgtcgtgcaacggcgaaaccaagtatttccgttgtgaagagaaaaacgggaacacgtcgtggaacgacacggtaacctgccccaacgcggagtgtcaacctctgcagttggagcacggctcttgtcagccggtgaaggaaaaatattccttcggcgagtacatgactataaactgtgatgtggggtacgaggttataggcgtatcctacattagctgcaccgctaatagttggaacgtcatcccctcgtgccagcagaaatgcgacattccgtctctgtcaaatggcctgatctccgggtcgaccttctcgataggtggggttattcatttgtcctgtaagagtgggttcactcttacaggctccccatcttcgacctgcatagatgggaagtggaaccccatccttcccacttgtgtcaggtcgaacgaggaattcgatccggtagatgacggccctgacgacgagacggatctgtcgaagctgtccaaagacgtggttcagtatgagcaggagatagaatctcttgaggctacttaccac

SEQ ID NO: 17 - RNA, 1593 nt, synthetic construct
  source 1..1593: mol_type = other RNA
agcaccacccagtacgaccacaaagagagctgcaacggcctgtactaccaaggctcttgttacatcctgcacagcgactataagagcttcgaggatgctaaggccaattgcgccgccgagagcagcacactgcctaacaagtccgacgtgctgaccacctggctgatcgactacgtggaagatacatggggaagcgacggcaaccccatcacaaaaaccacaagcgattatcaggacagcgacgtgtctcaggaggttagaaagtacttttgcaccgccgccgcctctatccagaccacagtgaacaccctgagcgagcggatcagctccaagctggagcaggaggcaaacgcaagcgcccagacaaagtgcgacatcgagatcggcaatttctacatcagacagaaccacggctgcaatatcaccgtgaagaatatgtgctccgccgacgcagatgcacagctggatgccgtgctgtccgccgcaaccgagacatactctggcctgacccctgagcagaaggcctatgtgccagccatgttcacagccgccctgaacatccagaccagcgtgaatacagtggtgcgggactttgagaactacgtgaagcagacctgcaattctagcgccgtggtggacaacaagctgaagatccagaatgtgatcatcgatgagtgttatggagcaccaggctcccctaccaacctggagttcatcaatacaggctcctctaagggcaactgcgccatcaaggccctgatgcagctgaccacaaaggccaccacacagatcgcacctaggcaggtggcaggcacgtgcacggtgcccacgatgaacaacgcgaagttgacgtccacggaaacctctttcaatgataaacaaaaagtcacgttcacatgtgactccggataccactctttggacccgaacgcagtttgtgaaacagataagtggaagtacgagaatccgtgcaagaaaatgtgcacggtgtcggattatgtatcagagttgtacgacaagccgttgtacgaggttaatagtaccatgaccttgtcgtgcaacggcgaaaccaagtatttccgttgtgaagagaaaaacgggaacacgtcgtggaacgacacggtaacctgccccaacgcggagtgtcaacctctgcagttggagcacggctcttctcagccggtgaaggaaaaatattccttcggcgagtacatgactataaactgtgatgtggggtacgaggttataggcgtatcctacattagctgcaccgctaatagttggaacgtcatcccctcgtgccagcagaaatgcgacattccgtctctgtcaaatggcctgatctccgggtcgaccttctcgataggtggggttattcatttgtcctgtaagagtgggttcactcttacaggctccccatcttcgacctgcatagatgggaagtggaaccccatccttcccacttgtgtcaggtcgaacgaggaattcgatccggtagatgacggccctgacgacgagacggatctgtcgaagctgtccaaagacgtggttcagtatgagcaggagatagaatctcttgaggctacttaccac

SEQ ID NO: 18 - DNA, 47 bp, synthetic construct
  source 1..47: mol_type = other DNA
gggaaataagagagaaaagaagagtaagaagaaatataagagccacc

SEQ ID NO: 19 - protein, 20 aa, synthetic construct
METDTLLLWVLLLWVPGSTG

SEQ ID NO: 20 - DNA, 60 bp, synthetic construct
  source 1..60: mol_type = other DNA
atggaaacagacaccctgctgctgtgggtcctgctgctctgggtgcctggcagcaccggc

SEQ ID NO: 21 - DNA, 110 bp, synthetic construct
  source 1..110: mol_type = other DNA
tgataataggctggagcctcggtggccatgcttcttgccccttgggcctccccccagcccctcctccccttcctgcacccgtacccccgtggtctttgaataaagtctga

SEQ ID NO: 22 - DNA, 276 bp, synthetic construct
  source 1..276: mol_type = other DNA
agcaccacccagtacgaccacaaagagagctgcaacggcctgtactaccaaggctcttgttacatcctgcacagcgactataagagcttcgaggatgctaaggccaattgcgccgccgagagcagcacactgcctaacaagtccgacgtgctgaccacctggctgatcgactacgtggaagatacatggggaagcgacggcaaccccatcacaaaaaccacaagcgattatcaggacagcgacgtgtctcaggaggttagaaagtacttttgcacc

SEQ ID NO: 23 - DNA, 537 bp, synthetic construct
  source 1..537: mol_type = other DNA
gccgccgcctctatccagaccacagtgaacaccctgagcgagcggatcagctccaagctggagcaggaggcaaacgcaagcgcccagacaaagtgcgacatcgagatcggcaatttctacatcagacagaaccacggctgcaatatcaccgtgaagaatatgtgctccgccgacgcagatgcacagctggatgccgtgctgtccgccgcaaccgagacatactctggcctgacccctgagcagaaggcctatgtgccagccatgttcacagccgccctgaacatccagaccagcgtgaatacagtggtgcgggactttgagaactacgtgaagcagacctgcaattctagcgccgtggtggacaacaagctgaagatccagaatgtgatcatcgatgagtgttatggagcaccaggctcccctaccaacctggagttcatcaatacaggctcctctaagggcaactgcgccatcaaggccctgatgcagctgaccacaaaggccaccacacagatcgcacctaggcaggtggcaggc

SEQ ID NO: 24 - DNA, 780 bp, synthetic construct
  source 1..780: mol_type = other DNA
acgtgcacggtgcccacgatgaacaacgcgaagttgacgtccacggaaacctctttcaatgataaacaaaaagtcacgttcacatgtgactccggataccactctttggacccgaacgcagtttgtgaaacagataagtggaagtacgagaatccgtgcaagaaaatgtgcacggtgtcggattatgtatcagagttgtacgacaagccgttgtacgaggttaatagtaccatgaccttgtcgtgcaacggcgaaaccaagtatttccgttgtgaagagaaaaacgggaacacgtcgtggaacgacacggtaacctgccccaacgcggagtgtcaacctctgcagttggagcacggctcttgtcagccggtgaaggaaaaatattccttcggcgagtacatgactataaactgtgatgtggggtacgaggttataggcgtatcctacattagctgcaccgctaatagttggaacgtcatcccctcgtgccagcagaaatgcgacattccgtctctgtcaaatggcctgatctccgggtcgaccttctcgataggtggggttattcatttgtcctgtaagagtgggttcactcttacaggctccccatcttcgacctgcatagatgggaagtggaaccccatccttcccacttgtgtcaggtcgaacgaggaattcgatccggtagatgacggccctgacgacgagacggatctgtcgaagctgtccaaagacgtggttcagtatgagcaggagatagaatctcttgaggctacttaccac

SEQ ID NO: 25 - RNA, 276 nt, synthetic construct
  source 1..276: mol_type = other RNA
agcaccacccagtacgaccacaaagagagctgcaacggcctgtactaccaaggctcttgttacatcctgcacagcgactataagagcttcgaggatgctaaggccaattgcgccgccgagagcagcacactgcctaacaagtccgacgtgctgaccacctggctgatcgactacgtggaagatacatggggaagcgacggcaaccccatcacaaaaaccacaagcgattatcaggacagcgacgtgtctcaggaggttagaaagtacttttgcacc

SEQ ID NO: 26 - RNA, 537 nt, synthetic construct
  source 1..537: mol_type = other RNA
gccgccgcctctatccagaccacagtgaacaccctgagcgagcggatcagctccaagctggagcaggaggcaaacgcaagcgcccagacaaagtgcgacatcgagatcggcaatttctacatcagacagaaccacggctgcaatatcaccgtgaagaatatgtgctccgccgacgcagatgcacagctggatgccgtgctgtccgccgcaaccgagacatactctggcctgacccctgagcagaaggcctatgtgccagccatgttcacagccgccctgaacatccagaccagcgtgaatacagtggtgcgggactttgagaactacgtgaagcagacctgcaattctagcgccgtggtggacaacaagctgaagatccagaatgtgatcatcgatgagtgttatggagcaccaggctcccctaccaacctggagttcatcaatacaggctcctctaagggcaactgcgccatcaaggccctgatgcagctgaccacaaaggccaccacacagatcgcacctaggcaggtggcaggc

SEQ ID NO: 27 - RNA, 780 nt, synthetic construct
  source 1..780: mol_type = other RNA
acgtgcacggtgcccacgatgaacaacgcgaagttgacgtccacggaaacctctttcaatgataaacaaaaagtcacgttcacatgtgactccggataccactctttggacccgaacgcagtttgtgaaacagataagtggaagtacgagaatccgtgcaagaaaatgtgcacggtgtcggattatgtatcagagttgtacgacaagccgttgtacgaggttaatagtaccatgaccttgtcgtgcaacggcgaaaccaagtatttccgttgtgaagagaaaaacgggaacacgtcgtggaacgacacggtaacctgccccaacgcggagtgtcaacctctgcagttggagcacggctcttgtcagccggtgaaggaaaaatattccttcggcgagtacatgactataaactgtgatgtggggtacgaggttataggcgtatcctacattagctgcaccgctaatagttggaacgtcatcccctcgtgccagcagaaatgcgacattccgtctctgtcaaatggcctgatctccgggtcgaccttctcgataggtggggttattcatttgtcctgtaagagtgggttcactcttacaggctccccatcttcgacctgcatagatgggaagtggaaccccatccttcccacttgtgtcaggtcgaacgaggaattcgatccggtagatgacggccctgacgacgagacggatctgtcgaagctgtccaaagacgtggttcagtatgagcaggagatagaatctcttgaggctacttaccac